European Patent Application EP 4 201 483 A1, published June 28, 2023. Title: LPL1 DERIVED IMMUNE ENHANCING PEPTIDES. Applicant: Eberhard Karls Universität Tübingen. The sequence listing filed with the application follows.

SEQUENCE LISTING (32 sequences)

SEQ ID NO: 1 - protein, 267 aa, Staphylococcus aureus
MKYKTERREAMGYLKRFALYISVMILIFAIAGCGKGNETKEDSKEEQIKKSFAITLDMYPIKNLEDLYDKEGYRDSEFKKGDKGMWTIYTDFAKSNKPGELDDEGMVLNLDRNTRTAKGHYFVTTFYRNGKLPDEKNYKIEMKNNKIILLDEVKDDKLKQKIENFKFFGQYANLKELRKYNNGDVSINENVPSYDVEYKMSNKDEIVKELRSRYNISTEKSPILKMHIDGDLKGSSVGYRKLEIDFSKRENSKLSVIEFLSYKPAKK

SEQ ID NO: 2 - protein, 64 aa, Staphylococcus aureus
TAKGHYFVTTFYRNGKLPDEKNYKIEMKNNKIILLDEVKDDKLKQKIENFKFFGQYANLKELRK

SEQ ID NO: 3 - protein, 9 aa, Staphylococcus aureus
GHYFVTTFY

SEQ ID NO: 4 - protein, 15 aa, Staphylococcus aureus
TAKGHYFVTTFYRNG

SEQ ID NO: 5 - protein, 271 aa, Staphylococcus hyicus
MMEYIKKIALYMSVLLLIIFIGGCENMKDEQKKEEQTNKTDSKEEQIKKSFAKTLDMYPIKNLEELYDKEGYRDGEFEKGDKGMWTIYTDFAKSNKPGELNDEGMVLNLDRNTRTAKGHYFVTTFYRNGKLPDEKNYKIEMKNNKIILLDEVKDDKLKQKIENFKFFGQYANLKELKKYNNGDVSINENVPSYDVEYKMSNKDEIVKELRSRYNISTEKSPILKMHIDGNLKGSSVGYRKLEIDFSKRENSKLSVIEFLSYKPAKVNNDER

SEQ ID NO: 6 - protein, 267 aa, Staphylococcus schweitzeri
MKYKTERREAMGYLKRFALYISVMILIFAIAGCGKGNETKEDSKEEQIKKSFAKTLDMYPIKNLEDLYDKEGYRDGEFKKGDKGMWTIYTDFAKSNKPGELNDEGMVLNLDRNTRTAKGHYFVTTFYRNGKLPDEKNYKIEMKNNKIILLDEVKDDKLKQKIENFKFFGQYANLKELKKYNNGDVSINENVPSYDVEYKMSNKDEIVKELRSSYNISTEKSPILKMHIDGHLKGSSVGYRKLEIDFSKRENSKLSVIEFLSYKPAKK

SEQ ID NO: 7 - protein, 277 aa, Staphylococcus argenteus
MRTINYDEKRGYGTMNNFRQYALCIGTSVLILLVSGCSGVSDTPEDSKETQIKKSFAKTLDMYPIKNLEDLYDKEGYRDGEFKKGDKGMWTIYTDFAKSNKPGELNDEGMVLNLDRNTRTAKGHYFVTTFYRNGKLPDEKNYKIEMKNNKIILLDEVKDDKLKQKIENFKFFGQYANLKELKKYNNADVSINENVPSYDVEYKMSNKDEIVKELRRRYNISTEKSPILKMHIDGDLKGSSVGYRKLEIDFSKRENSKLSVIEFLSYKPAKNSIDKEY

SEQ ID NO: 8 - protein, 170 aa, Listeria monocytogenes
NEGMVLYLDRNTRTAKGHYFVKTFYNKGKFPDRKNYKVEMKNNKIILLDKVEDTNLKKRIENFKFFGQYANLKELKNYNNGDVSINENVPSYDAKFKMSNKDENVKQLRSRYNIPTDKAPVLKMHIDGNLKGSSVGDRKLEIDFSKRENSHLSVIDSLDYQPAKVDEDER

SEQ ID NO: 9 - protein, 130 aa, Lactobacillus ruminis
MKSIKRIGLCISLLILSIFVTSCDGDNKITGDSKETQIKKSFSKTLDMYPIKNLEDLYDKEGYRDSEFKKGDKGMWTIYTDFAKSNKPGELSNEGMVLYLDRNTRTAKGYYFVRTFYRKDKLPDRKNYKV

SEQ ID NO: 10 - protein, 271 aa, Escherichia coli
MMGYIKRMALYMSVFLLIIFIVGCRNMKDEQKKEEQTNKTDSKEEQIKKSFEKTLDMYPIKNLEELYDKEGYRDGEFKKGDKGMWTIYTDFAKSNKQGGLSNEGMVLYLDRNTRTAKGHYFVKTFYNKGKFPDRKNYKVEMKNNKIILLDKVEDTNLKKRIENFKFFGQYANLKELKNYNNGDVSINENVPSYDAKFKMSNKDENVKQLRSRYNIPTDKAPVLKMHIDGNLKGSSVGYKKLEIDFSKGGKSDLSVIDSLNFQPAKVDEDDE

SEQ ID NO: 11 - protein, 137 aa, Klebsiella pneumoniae
MGYLKRFSLYISVMILIFAIAGCGKGNETKEDSKEEQIKKSFAKTVDMYPIKNLEDLYDKEGYRDGEFKKGDKGMWTIYTDFAKSNKPGELSNEGMVLYLDRNTRTAKGYYFVRTFYRKDKLPDRKNYKVEMKNNKI

SEQ ID NO: 12 - protein, 194 aa, Pseudomonas aeruginosa
MEYIKKIALYMSVLLLIIFIGGCENMKDEQKKEEQTNKTDSKEEQIKKSFAKTLDMYPIKNLEELYDKEGYRDGEFEKGDKGMWTIYTDFAKSNKPGELNDEGMVLNLDRNTRTAKGHYFVTTFYRNGKLPDEKNYKIEMKNNKIILLDEVKDDKLKQKIENFKFFGQYANLKELKKYNNGDVSINENVPSYDV

SEQ ID NO: 13 - protein, 15 aa, Staphylococcus hyicus
TAKGHYFVTTFYRNG

SEQ ID NO: 14 - protein, 15 aa, Staphylococcus schweitzeri
TAKGHYFVTTFYRNG

SEQ ID NO: 15 - protein, 15 aa, Staphylococcus argenteus
TAKGHYFVTTFYRNG

SEQ ID NO: 16 - protein, 15 aa, Listeria monocytogenes
TAKGHYFVKTFYNKG

SEQ ID NO: 17 - protein, 13 aa, Lactobacillus ruminis
TAKGYYFVRTFYR

SEQ ID NO: 18 - protein, 15 aa, Escherichia coli
TAKGHYFVKTFYNKG

SEQ ID NO: 19 - protein, 13 aa, Klebsiella pneumoniae
TAKGYYFVRTFYR

SEQ ID NO: 20 - protein, 15 aa, Pseudomonas aeruginosa
TAKGHYFVTTFYRNG

SEQ ID NO: 21 - protein, 9 aa, Staphylococcus hyicus
GHYFVTTFY

SEQ ID NO: 22 - protein, 9 aa, Staphylococcus schweitzeri
GHYFVTTFY

SEQ ID NO: 23 - protein, 9 aa, Staphylococcus argenteus
GHYFVTTFY

SEQ ID NO: 24 - protein, 9 aa, Listeria monocytogenes
GHYFVKTFY

SEQ ID NO: 25 - protein, 9 aa, Lactobacillus ruminis
GYYFVRTFY

SEQ ID NO: 26 - protein, 9 aa, Escherichia coli
GHYFVKTFY

SEQ ID NO: 27 - protein, 9 aa, Klebsiella pneumoniae
GYYFVRTFY

SEQ ID NO: 28 - protein, 9 aa, Pseudomonas aeruginosa
GHYFVTTFY

SEQ ID NO: 29 - protein, 67 aa, Staphylococcus aureus
DSKEEQIKKSFAITLDMYPIKNLEDLYDKEGYRDSEFKKGDKGMWTIYTDFAKSNKPGELDDEGMVL

SEQ ID NO: 30 - protein, 64 aa, Staphylococcus aureus
DEIVKELRSRYNISTEKSPILKMHIDGDLKGSSVGYRKLEIDFSKRENSKLSVIEFLSYKPAKK

SEQ ID NO: 31 - protein, 38 aa, Staphylococcus aureus
RSRYNISTEKSPILKMHIDGDLKGSSVGYRKLEIDFSK

SEQ ID NO: 32 - protein, 15 aa, Staphylococcus aureus
DEIVKELRSRYNIST